European Patent Application EP 4 549 577 A1, published May 7, 2025. Title: NOVEL INDUCED CYTOPLASMIC IVT (ICIVT)-LIKE COMPOSITION AND THE RELATED VACCINE MEDICINE DESIGNS THEREOF. Applicant: MELLO BIOTECH TAIWAN CO., LTD. The sequence listing filed with the application follows.

SEQUENCE LISTING (21 sequences)

SEQ ID NO: 1-2 - skipped (2 entries)

SEQ ID NO: 3 - RNA, 73 nt, synthetic construct
  source 1..73: mol_type = other RNA
  misc_difference 3: note = May be thymine
  misc_difference 7: note = May be thymine
  misc_difference 8: note = May be thymine
  misc_difference 13: note = May be thymine
  misc_difference 14: note = May be thymine
  misc_difference 15: note = May be thymine
  misc_difference 20: note = May be thymine
  misc_difference 26: note = May be thymine
  misc_difference 29: note = May be thymine
  misc_difference 30: note = May be thymine
  misc_difference 31: note = May be thymine
  misc_difference 33: note = May be thymine
  misc_difference 35: note = May be thymine
  misc_difference 39: note = May be thymine
  misc_difference 40: note = May be thymine
  misc_difference 41: note = May be thymine
  misc_difference 47: note = May be thymine
  misc_difference 51: note = May be thymine
  misc_difference 54: note = May be thymine
  misc_difference 55: note = May be thymine
  misc_difference 59: note = May be thymine
  misc_difference 61: note = May be thymine
  misc_difference 62: note = May be thymine
  misc_difference 63: note = May be thymine
  misc_difference 64: note = May be thymine
  misc_difference 67: note = May be thymine
  misc_difference 73: note = May be thymine
gctcccttcaactttaacatggaagtgctttctgtgactttaaaagtaagtgcttccatgttttagtaggagt

SEQ ID NO: 4 - RNA, 68 nt, synthetic construct
  source 1..68: mol_type = other RNA
  misc_difference 3: note = May be thymine
  misc_difference 4: note = May be thymine
  misc_difference 5: note = May be thymine
  misc_difference 8: note = May be thymine
  misc_difference 9: note = May be thymine
  misc_difference 10: note = May be thymine
  misc_difference 15: note = May be thymine
  misc_difference 21: note = May be thymine
  misc_difference 25: note = May be thymine
  misc_difference 28: note = May be thymine
  misc_difference 30: note = May be thymine
  misc_difference 32: note = May be thymine
  misc_difference 43: note = May be thymine
  misc_difference 47: note = May be thymine
  misc_difference 50: note = May be thymine
  misc_difference 51: note = May be thymine
  misc_difference 55: note = May be thymine
  misc_difference 57: note = May be thymine
  misc_difference 58: note = May be thymine
  misc_difference 59: note = May be thymine
  misc_difference 63: note = May be thymine
cctttgctttaacatgggggtacctgctgtgtgaaacaaaagtaagtgcttccatgtttcagtggagg

SEQ ID NO: 5 - RNA, 69 nt, synthetic construct
  source 1..69: mol_type = other RNA
  misc_difference 8: note = May be thymine
  misc_difference 9: note = May be thymine
  misc_difference 15: note = May be thymine
  misc_difference 19: note = May be thymine
  misc_difference 21: note = May be thymine
  misc_difference 24: note = May be thymine
  misc_difference 25: note = May be thymine
  misc_difference 28: note = May be thymine
  misc_difference 29: note = May be thymine
  misc_difference 30: note = May be thymine
  misc_difference 36: note = May be thymine
  misc_difference 44: note = May be thymine
  misc_difference 48: note = May be thymine
  misc_difference 51: note = May be thymine
  misc_difference 52: note = May be thymine
  misc_difference 56: note = May be thymine
  misc_difference 58: note = May be thymine
  misc_difference 59: note = May be thymine
  misc_difference 60: note = May be thymine
  misc_difference 61: note = May be thymine
  misc_difference 64: note = May be thymine
  misc_difference 67: note = May be thymine
ccaccacttaaacgtggatgtacttgctttgaaactaaagaagtaagtgcttccatgttttggtgatgg

SEQ ID NO: 6 - RNA, 68 nt, synthetic construct
  source 1..68: mol_type = other RNA
  misc_difference 3: note = May be thymine
  misc_difference 5: note = May be thymine
  misc_difference 8: note = May be thymine
  misc_difference 9: note = May be thymine
  misc_difference 10: note = May be thymine
  misc_difference 15: note = May be thymine
  misc_difference 24: note = May be thymine
  misc_difference 25: note = May be thymine
  misc_difference 28: note = May be thymine
  misc_difference 30: note = May be thymine
  misc_difference 35: note = May be thymine
  misc_difference 44: note = May be thymine
  misc_difference 48: note = May be thymine
  misc_difference 51: note = May be thymine
  misc_difference 52: note = May be thymine
  misc_difference 56: note = May be thymine
  misc_difference 58: note = May be thymine
  misc_difference 59: note = May be thymine
  misc_difference 60: note = May be thymine
  misc_difference 64: note = May be thymine
  misc_difference 66: note = May be thymine
cctctactttaacatggaggcacttgctgtgacatgacaaaaataagtgcttccatgtttgagtgtgg

SEQ ID NO: 7 - RNA, 44 nt, synthetic construct
  source 1..44: mol_type = other RNA
  misc_difference 2: note = May be thymine
  misc_difference 4: note = May be thymine
  misc_difference 6: note = May be thymine
  misc_difference 10: note = May be thymine
  misc_difference 12: note = May be thymine
  misc_difference 16: note = May be thymine
  misc_difference 21: note = May be thymine
  misc_difference 25: note = May be thymine
  misc_difference 28: note = May be thymine
  misc_difference 29: note = May be thymine
  misc_difference 32: note = May be thymine
  misc_difference 37: note = May be thymine
ctgtgtggctgtcactcggctgcatgcttagtgcactcacgcag

SEQ ID NO: 8 - RNA, 65 nt, synthetic construct
  source 1..65: mol_type = other RNA
  misc_difference 2: note = May be thymine
  misc_difference 4: note = May be thymine
  misc_difference 6: note = May be thymine
  misc_difference 10: note = May be thymine
  misc_difference 12: note = May be thymine
  misc_difference 16: note = May be thymine
  misc_difference 21: note = May be thymine
  misc_difference 25: note = May be thymine
  misc_difference 28: note = May be thymine
  misc_difference 29: note = May be thymine
  misc_difference 32: note = May be thymine
  misc_difference 37: note = May be thymine
  misc_difference 45: note = May be thymine
  misc_difference 47: note = May be thymine
  misc_difference 50: note = May be thymine
  misc_difference 51: note = May be thymine
  misc_difference 54: note = May be thymine
  misc_difference 58: note = May be thymine
  misc_difference 61: note = May be thymine
  misc_difference 62: note = May be thymine
  misc_difference 65: note = May be thymine
ctgtgtggctgtcactcggctgcatgcttagtgcactcacgcagtataattaataactaattact

SEQ ID NO: 9 - RNA, 147 nt, synthetic construct
  source 1..147: mol_type = other RNA
  misc_difference 2: note = May be thymine
  misc_difference 5: note = May be thymine
  misc_difference 6: note = May be thymine
  misc_difference 20: note = May be thymine
  misc_difference 24: note = May be thymine
  misc_difference 27: note = May be thymine
  misc_difference 29: note = May be thymine
  misc_difference 31: note = May be thymine
  misc_difference 33: note = May be thymine
  misc_difference 34: note = May be thymine
  misc_difference 36: note = May be thymine
  misc_difference 43: note = May be thymine
  misc_difference 46: note = May be thymine
  misc_difference 47: note = May be thymine
  misc_difference 52: note = May be thymine
  misc_difference 53: note = May be thymine
  misc_difference 54: note = May be thymine
  misc_difference 57: note = May be thymine
  misc_difference 61: note = May be thymine
  misc_difference 63: note = May be thymine
  misc_difference 64: note = May be thymine
  misc_difference 73: note = May be thymine
  misc_difference 76: note = May be thymine
  misc_difference 84: note = May be thymine
  misc_difference 86: note = May be thymine
  misc_difference 90: note = May be thymine
  misc_difference 91: note = May be thymine
  misc_difference 92: note = May be thymine
  misc_difference 95: note = May be thymine
  misc_difference 101: note = May be thymine
  misc_difference 103: note = May be thymine
  misc_difference 114: note = May be thymine
  misc_difference 119: note = May be thymine
  misc_difference 128: note = May be thymine
  misc_difference 129: note = May be thymine
  misc_difference 131: note = May be thymine
  misc_difference 135: note = May be thymine
  misc_difference 138: note = May be thymine
  misc_difference 139: note = May be thymine
  misc_difference 140: note = May be thymine
gtcgttgacaggacacgagtaactcgtctatcttctgcaggctgcttacggtttcgtccgtgttgcagccgatcatcagcacatctaggtttcgtccgggtgtgaccgaaaggtaagatggagagccttgtccctggtttcaacgag

SEQ ID NO: 10 - RNA, 88 nt, synthetic construct
  source 1..88: mol_type = other RNA
  misc_difference 3: note = May be thymine
  misc_difference 4: note = May be thymine
  misc_difference 6: note = May be thymine
  misc_difference 10: note = May be thymine
  misc_difference 11: note = May be thymine
  misc_difference 18: note = May be thymine
  misc_difference 21: note = May be thymine
  misc_difference 22: note = May be thymine
  misc_difference 23: note = May be thymine
  misc_difference 24: note = May be thymine
  misc_difference 31: note = May be thymine
  misc_difference 35: note = May be thymine
  misc_difference 36: note = May be thymine
  misc_difference 38: note = May be thymine
  misc_difference 42: note = May be thymine
  misc_difference 43: note = May be thymine
  misc_difference 48: note = May be thymine
  misc_difference 49: note = May be thymine
  misc_difference 51: note = May be thymine
  misc_difference 57: note = May be thymine
  misc_difference 59: note = May be thymine
  misc_difference 60: note = May be thymine
  misc_difference 63: note = May be thymine
  misc_difference 64: note = May be thymine
  misc_difference 66: note = May be thymine
  misc_difference 71: note = May be thymine
  misc_difference 72: note = May be thymine
  misc_difference 75: note = May be thymine
  misc_difference 78: note = May be thymine
  misc_difference 81: note = May be thymine
  misc_difference 82: note = May be thymine
  misc_difference 84: note = May be thymine
  misc_difference 87: note = May be thymine
  misc_difference 88: note = May be thymine
aattataaattaccagatgattttacaggctgcgttatagcttggaattctaacaatcttgattctaaggttggtggtaattataatt

SEQ ID NO: 11 - RNA, 129 nt, synthetic construct
  source 1..129: mol_type = other RNA
  misc_difference 7: note = May be thymine
  misc_difference 9: note = May be thymine
  misc_difference 10: note = May be thymine
  misc_difference 17: note = May be thymine
  misc_difference 21: note = May be thymine
  misc_difference 39: note = May be thymine
  misc_difference 42: note = May be thymine
  misc_difference 43: note = May be thymine
  misc_difference 44: note = May be thymine
  misc_difference 46: note = May be thymine
  misc_difference 47: note = May be thymine
  misc_difference 53: note = May be thymine
  misc_difference 55: note = May be thymine
  misc_difference 58: note = May be thymine
  misc_difference 59: note = May be thymine
  misc_difference 60: note = May be thymine
  misc_difference 61: note = May be thymine
  misc_difference 70: note = May be thymine
  misc_difference 76: note = May be thymine
  misc_difference 77: note = May be thymine
  misc_difference 83: note = May be thymine
  misc_difference 86: note = May be thymine
  misc_difference 90: note = May be thymine
  misc_difference 91: note = May be thymine
  misc_difference 94: note = May be thymine
  misc_difference 102: note = May be thymine
  misc_difference 104: note = May be thymine
  misc_difference 107: note = May be thymine
  misc_difference 110: note = May be thymine
  misc_difference 111: note = May be thymine
  misc_difference 115: note = May be thymine
  misc_difference 116: note = May be thymine
  misc_difference 119: note = May be thymine
  misc_difference 122: note = May be thymine
  misc_difference 124: note = May be thymine
  misc_difference 125: note = May be thymine
  misc_difference 128: note = May be thymine
cacaaatattaccagatccatcaaaaccaagcaagaggtcatttattgaagatctacttttcaacaaagtgacacttgcagatgctggcttcatcaaacaatatggtgattgccttggtgatattgctg

SEQ ID NO: 12 - RNA, 189 nt, synthetic construct
  source 1..189: mol_type = other RNA
  misc_difference 8: note = May be thymine
  misc_difference 10: note = May be thymine
  misc_difference 13: note = May be thymine
  misc_difference 15: note = May be thymine
  misc_difference 16: note = May be thymine
  misc_difference 19: note = May be thymine
  misc_difference 20: note = May be thymine
  misc_difference 22: note = May be thymine
  misc_difference 26: note = May be thymine
  misc_difference 31: note = May be thymine
  misc_difference 32: note = May be thymine
  misc_difference 33: note = May be thymine
  misc_difference 34: note = May be thymine
  misc_difference 41: note = May be thymine
  misc_difference 42: note = May be thymine
  misc_difference 45: note = May be thymine
  misc_difference 49: note = May be thymine
  misc_difference 50: note = May be thymine
  misc_difference 56: note = May be thymine
  misc_difference 59: note = May be thymine
  misc_difference 62: note = May be thymine
  misc_difference 64: note = May be thymine
  misc_difference 65: note = May be thymine
  misc_difference 66: note = May be thymine
  misc_difference 67: note = May be thymine
  misc_difference 68: note = May be thymine
  misc_difference 70: note = May be thymine
  misc_difference 72: note = May be thymine
  misc_difference 73: note = May be thymine
  misc_difference 74: note = May be thymine
  misc_difference 78: note = May be thymine
  misc_difference 79: note = May be thymine
  misc_difference 83: note = May be thymine
  misc_difference 85: note = May be thymine
  misc_difference 86: note = May be thymine
  misc_difference 87: note = May be thymine
  misc_difference 91: note = May be thymine
  misc_difference 92: note = May be thymine
  misc_difference 93: note = May be thymine
  misc_difference 97: note = May be thymine
  misc_difference 98: note = May be thymine
  misc_difference 105: note = May be thymine
  misc_difference 109: note = May be thymine
  misc_difference 112: note = May be thymine
  misc_difference 126: note = May be thymine
  misc_difference 128: note = May be thymine
  misc_difference 140: note = May be thymine
  misc_difference 142: note = May be thymine
  misc_difference 144: note = May be thymine
  misc_difference 149: note = May be thymine
  misc_difference 150: note = May be thymine
  misc_difference 151: note = May be thymine
  misc_difference 152: note = May be thymine
  misc_difference 153: note = May be thymine
  misc_difference 158: note = May be thymine
  misc_difference 159: note = May be thymine
  misc_difference 162: note = May be thymine
  misc_difference 163: note = May be thymine
  misc_difference 166: note = May be thymine
  misc_difference 176: note = May be thymine
  misc_difference 183: note = May be thymine
  misc_difference 184: note = May be thymine
  misc_difference 185: note = May be thymine
  misc_difference 188: note = May be thymine
gcaaaaatgtgatcttgcttgtaaatacaattttgagaggttaataaattacaagtagtgctatttttgtatttaggttagctatttagctttacgttccaggatgcctagtggcagccccacaatatccaggaagccctctctgcggtttttcagattcgttagtcgaaaaacctaagaaatttaatg

SEQ ID NO: 13 - RNA, 294 nt, synthetic construct
  source 1..294: mol_type = other RNA
  misc_difference 4: note = May be thymine
  misc_difference 9: note = May be thymine
  misc_difference 11: note = May be thymine
  misc_difference 18: note = May be thymine
  misc_difference 21: note = May be thymine
  misc_difference 23: note = May be thymine
  misc_difference 25: note = May be thymine
  misc_difference 26: note = May be thymine
  misc_difference 40: note = May be thymine
  misc_difference 42: note = May be thymine
  misc_difference 48: note = May be thymine
  misc_difference 53: note = May be thymine
  misc_difference 54: note = May be thymine
  misc_difference 57: note = May be thymine
  misc_difference 59: note = May be thymine
  misc_difference 63: note = May be thymine
  misc_difference 65: note = May be thymine
  misc_difference 68: note = May be thymine
  misc_difference 75: note = May be thymine
  misc_difference 89: note = May be thymine
  misc_difference 103: note = May be thymine
  misc_difference 106: note = May be thymine
  misc_difference 109: note = May be thymine
  misc_difference 111: note = May be thymine
  misc_difference 122: note = May be thymine
  misc_difference 126: note = May be thymine
  misc_difference 136: note = May be thymine
  misc_difference 137: note = May be thymine
  misc_difference 153: note = May be thymine
  misc_difference 156: note = May be thymine
  misc_difference 157: note = May be thymine
  misc_difference 158: note = May be thymine
  misc_difference 160: note = May be thymine
  misc_difference 161: note = May be thymine
  misc_difference 165: note = May be thymine
  misc_difference 174: note = May be thymine
  misc_difference 178: note = May be thymine
  misc_difference 182: note = May be thymine
  misc_difference 188: note = May be thymine
  misc_difference 189: note = May be thymine
  misc_difference 190: note = May be thymine
  misc_difference 196: note = May be thymine
  misc_difference 210: note = May be thymine
  misc_difference 213: note = May be thymine
  misc_difference 221: note = May be thymine
  misc_difference 224: note = May be thymine
  misc_difference 226: note = May be thymine
  misc_difference 227: note = May be thymine
  misc_difference 231: note = May be thymine
  misc_difference 243: note = May be thymine
  misc_difference 244: note = May be thymine
  misc_difference 246: note = May be thymine
  misc_difference 249: note = May be thymine
  misc_difference 252: note = May be thymine
  misc_difference 256: note = May be thymine
  misc_difference 259: note = May be thymine
  misc_difference 263: note = May be thymine
  misc_difference 266: note = May be thymine
  misc_difference 267: note = May be thymine
  misc_difference 273: note = May be thymine
  misc_difference 285: note = May be thymine
  misc_difference 287: note = May be thymine
  misc_difference 290: note = May be thymine
cactcccctgtgaggactactgtcttcacgcagaaagcgtctagccatggcgttagtatgagtgtcgtgcagcctccaggaccccccctcccgggagagccatagtggtctgcggaaccggtgagtacaccggaattgccaggacgaccgggtcctttcttggatcaacccgctcaatgcctggagatttgggcgtgcccccgcgagactgctagccgagtagtgttgggtcgcgaaaggccttgtggtactgcctgatgggtgcttgcgagtgccccgggaggtctcgtagac

SEQ ID NO: 14 - RNA, 55 nt, synthetic construct
  source 1..55: mol_type = other RNA
  misc_difference 10: note = May be thymine
  misc_difference 14: note = May be thymine
  misc_difference 17: note = May be thymine
  misc_difference 19: note = May be thymine
  misc_difference 21: note = May be thymine
  misc_difference 23: note = May be thymine
  misc_difference 24: note = May be thymine
  misc_difference 26: note = May be thymine
  misc_difference 33: note = May be thymine
  misc_difference 36: note = May be thymine
  misc_difference 37: note = May be thymine
  misc_difference 42: note = May be thymine
  misc_difference 43: note = May be thymine
  misc_difference 44: note = May be thymine
  misc_difference 47: note = May be thymine
  misc_difference 51: note = May be thymine
  misc_difference 53: note = May be thymine
  misc_difference 54: note = May be thymine
ggacacgagtaactcgtctatcttctgcaggctgcttacggtttcgtccgtgttg

SEQ ID NO: 15 - RNA, 52 nt, synthetic construct
  source 1..52: mol_type = other RNA
  misc_difference 8: note = May be thymine
  misc_difference 11: note = May be thymine
  misc_difference 19: note = May be thymine
  misc_difference 21: note = May be thymine
  misc_difference 25: note = May be thymine
  misc_difference 26: note = May be thymine
  misc_difference 27: note = May be thymine
  misc_difference 28: note = May be thymine
  misc_difference 30: note = May be thymine
  misc_difference 36: note = May be thymine
  misc_difference 38: note = May be thymine
  misc_difference 49: note = May be thymine
cagccgatcatcagcacatctaggttttgtccgggtgtgaccgaaaggtaag

SEQ ID NO: 16 - DNA, 23 bp, synthetic construct
  source 1..23: mol_type = other DNA
cagttccaattgtgaagattctc

SEQ ID NO: 17 - DNA, 20 bp, synthetic construct
  source 1..20: mol_type = other DNA
cttgatgacgttctcagtgc

SEQ ID NO: 18 - DNA, 54 bp, synthetic construct
  source 1..54: mol_type = other DNA
gatatctaatacgactcactatagggagaggtgccaccatggtacttggtagtt

SEQ ID NO: 19 - DNA, 59 bp, synthetic construct
  source 1..59: mol_type = other DNA
gatatctaatacgactcactatagggagactagtggccaccatgttcttgttaacaact

SEQ ID NO: 20 - DNA, 48 bp, synthetic construct
  source 1..48: mol_type = other DNA
gatatctaatacgactcactatagggagaggtatggtacttggtagtt

SEQ ID NO: 21 - DNA, 25 bp, synthetic construct
  source 1..25: mol_type = other DNA
tctaatacgactcactatagggaga